European Patent Specification EP 3 773 524 B1, published April 9, 2025. Title: LASOFOXIFENE TREATMENT OF BREAST CANCER. Applicant: DUKE UNIVERSITY. The sequence listing filed with the application follows.

SEQUENCE LISTING (8 sequences)

SEQ ID NO: 1 - DNA, 21 bp, Artificial Sequence
  Description of Artificial Sequence: Synthetic primer
aatgacctgctgctggagatg

SEQ ID NO: 2 - DNA, 21 bp, Artificial Sequence
  Description of Artificial Sequence: Synthetic primer
gaggggcaccacgttcttgca

SEQ ID NO: 3 - DNA, 21 bp, Artificial Sequence
  Description of Artificial Sequence: Synthetic primer
gacctgctgctggagatgctg

SEQ ID NO: 4 - DNA, 21 bp, Artificial Sequence
  Description of Artificial Sequence: Synthetic primer
gctgaggggcaccacgttctt

SEQ ID NO: 5 - DNA, 21 bp, Artificial Sequence
  Description of Artificial Sequence: Synthetic primer
tgtgacctgctgctggagatg

SEQ ID NO: 6 - DNA, 21 bp, Artificial Sequence
  Description of Artificial Sequence: Synthetic primer
gctgaggggcaccacgttctt

SEQ ID NO: 7 - DNA, 21 bp, Artificial Sequence
  Description of Artificial Sequence: Synthetic primer
ggtctgctgctggagatgctg

SEQ ID NO: 8 - DNA, 21 bp, Artificial Sequence
  Description of Artificial Sequence: Synthetic primer
atagaggggcaccacgttctt